European Patent Specification EP 3 394 289 B1, published March 26, 2025. Title: MICROBIAL MARKER IN SPONDYLOARTHRITIS. Applicant: VIB VZW UNIVERSITEIT GENT KATHOLIEKE UNIVERSITEIT LEUVEN, K.U.LEUVEN R&D. The sequence listing filed with the application follows.

SEQUENCE LISTING (26 sequences)

SEQ ID NO: 1 - DNA, 252 bp, Dialister micraerophilus
tacgtaggtggcaagcgttgtccggaattattgggcgtaaagcgcgcgcaggcggcttcttaagtccatcttaaaagtgcggggcttaaccccgtgatgggatggaaactgggaggctggagtatcggagaggaaagtggaattcctagtgtagcggtgaaatgcgtagagattaggaagaacaccggtggcgaaggcgactttctggacgacaactgacgctgaggcgcgaaagcgtggggagcaaacagg

SEQ ID NO: 2 - DNA, 252 bp, Dialister succinatiphilus
tacgtaggtggcaagcgttgtccggaattattgggcgtaaagcgcgcgcaggcggctttctaagtccatcttaaaagtgcggggcttaaccccgtgatgggatggaaactggaaagctggagtatcggagaggaaagtggaattcctagtgtagcggtgaaatgcgtagagattaggaagaacaccggtggcgaaggcgactttctggacgacaactgacgttgaggcacgaaagcgtgggtatcgaacagg

SEQ ID NO: 3 - DNA, 252 bp, Dialister sp.
tacgtatggtgcaagcgttgtccggaattattgggcgtaaagcgcgcgcaggcggctttctaagtccatcttaaaagtgcggggcttaaccccgtgatgggaaggaaactgggaagctggagtatcggagaggaaagtggaattcctagtgtagcggtgaaatgcgtagagattaggaagaacaccggtggcgaaggcgactttctggacgaaaactgacgctgaggcgcgaaagcgtggggagcaaacagg

SEQ ID NO: 4 - DNA, 252 bp, Dialister invisus
aacgtaggtcacaagcgttgtccggaattattgggcgtaaagcgcgcgcaggcggcttcccaagtccctcttaaaagtgcggggcttaaccccgtgatgggaaggaaactgggaagctggagtatcggagaggaaagtggaattcctagtgtagcggtgaaatgcgtagagattaggaagaacaccggtggcgaaggcgactttctggacgaaaactgacgctgaggcgcgaaagcgtggggagcaaacagg

SEQ ID NO: 5 - DNA, 252 bp, Dialister invisus
tacgtaggtggcaagcgttgtccggaattattgggcgtaaagcgcgcgcaggcggcttcccaagtccctcttaaaagtgcggggcttaaccccgtgatgggaaggaaactgggaagctggagtatcggagaggaaagtggaattcctagtgtagcggtgaaatgcgtagagattaggaagaacaccggtggcgaaggcgactttctggacgaaaactgacgctgaggcgcgaaagtgcgggtatcgaacagg

SEQ ID NO: 6 - DNA, 272 bp, Dialister invisus
agtgtcagccgccgcggtaatacgtaggtggcaagcgttgtccggaattattgggcgtaaagcgcgcgcaggcggcttcccaagtccctcttaaaagtgcggggcttaaccccgtgatgggaaggaaactgggaagctggagtatcggagaggaaagtggaattcctagtgtagcggtgaaatgcgtagagattaggaagaacaccggtggcgaaggcgactttctggacgaaaactgacgctgaggcgcgaaagcgtggggagcaaacagg

SEQ ID NO: 7 - DNA, 249 bp, Dialister invisus
acgtaggtggcaagcgttgtccggaattattgggcgtaaagcgcgcgcaggcggcttcccaagtccctcttaaaagtgcggggcttaaccccgtgagggaaggaaactgggaagctggagtatcggagaggaaagtggaattcctagtgtagcggtgaaatgcgtagagattaggaagaacaccggtggcgaaggcgactttctggacgaaaactgacgctgaggcgcgaaagcgtggggagcaaacag

SEQ ID NO: 8 - DNA, 250 bp, Dialister sp.
acgtaggtggcaagcgttgtccggaattattgggcgtaaagcgcgcgcaggcggcttcccaagtccctcttaaaagtgcggggcttaaccccgtgatgggaaggaaactgggaagctggagtatcggagaggaaagtggaattcctagtgtagcggtgaaatgcgtagatattaggaggaacaccagtggcgaaggcggcttactggacagtaactgacgttgaggctcgaaagcgtggggagcaaacag

SEQ ID NO: 9 - DNA, 252 bp, Dialister invisus
cctgtttgctccccacgctttcgtgcctcagtgtcagtagcagtccagtaagtcgccttcgccactggtgttcctcctaatatctacgcatttcaccgctacactaggaattccacttacctctccgatactccagcttcccagtttccttcccatcacggggttaagccccgcacttttaagagggacttgggaagccgcctgcgcgcgctttacgcccaataattccggacaacgcttgccacctacgta

SEQ ID NO: 10 - DNA, 252 bp, Dialister propionifaciens
cctgtttgctccccacgctttcgtgcctcagtgtcagtagcagtccagtaagtcgccttcgccactggtgttcttcctaatctctacgcatttcaccgctacactaggaattccactttcctctccgatactccagcctctcagtttccatcccatcacggggttaagccccgcacttttaagatggacttaagaagccgcctgcgcgcgctttacgcccaataattccggacaacgcttgccacctacgta

SEQ ID NO: 11 - DNA, 252 bp, Dialister sp.
cctgtttgctccccacgctttcgcgcctcagcgtcagttttcgtccagaaagtcgccttcgccaccggtgttcttcctaatatctacgcatttcaccgctacactaggaattccaccttcctctccgatactccagtctcccagtttccatcccctcacggggttaagccccgcacttctaagatagacttaagagaccgcctgcgcgcgctttacgcccaataattccggacaacgcttgccacctacgta

SEQ ID NO: 12 - DNA, 252 bp, Dialister invisus
cctgttcgctcccctagctttcgcgcctcagcgtcagtggcggcccagaaggctgccttcgccatcggtgttcttcccaatatctgcgcatttcaccgctacactgggaattccactttcctctccgatactccagcttcccagtttccttcccatcacggggttaagccccgcacttttaagagggacttgggaagccgcctgcgcgcgctttacgcccaataattccggacaacgcttgccacctacgta

SEQ ID NO: 13 - DNA, 252 bp, Dialister invisus
cctgtttgatacccacactttcgagcctcaatgtcagttgcagcttagcaggctgccttcgcaatcggagttcttcgtgatatctaagcatttcaccgctacactaggaattccactttcctctccgatactccagcttcccagtttccttcccatcacggggttaagccccgcacttttaagagggacttgggaagccgcctgcgcgcgctttacgcccaataattccggacaacgcttgccacctacgta

SEQ ID NO: 14 - DNA, 252 bp, Dialister invisus
cctgtttgctccccacactttcgcgcctcagcgtcagttacagtccagttagtcgccttcgccactggtgttcctcccaatctctacgcatttcaccgctacactgggaattccactaacctctccgatactccagcttcccagtttccttcccatcacggggttaagccccgcacttttaagagggacttgggaagccgcctgcgcgcgctttacgcccaataattccggacaacgcttgccacctacgta

SEQ ID NO: 15 - DNA, 252 bp, Dialister invisus
cctgttcgctccccacgctttcgagcctcagcgtcagttacagaccagagagccgctttcgccaccggtgttcctccatatatctacgcatttcaccgctacacatggaattccactttcctctccgatactccagcttcccagtttccttcccatcacggggttaagccccgcacttttaagagggacttgggaagccgcctgcgcgcgctttacgcccaataattccggacaacgcttgccacctacgta

SEQ ID NO: 16 - DNA, 252 bp, Dialister succinatiphilus
cctgtttgctccccacgctttcgcgcctcagcgtcagttgtcgtccagaaagccgccttcgccaccggtgttcttcctaatctctacgcatttcaccgctacactaggaattccgctttcctctccgatactccagctcttcagtttccatcccatcatggggttaagccccacgcttttaagatggacttaaagggccgcctgcgcgcgctttacgcccaataattccggacaacgcttgccacctacgta

SEQ ID NO: 17 - DNA, 252 bp, Dialister propionifaciens
cctgtttgctccccacgctttcgagcctcagcgtcagttatcgtccagtaagccgccttcgccactggtgttcctcctaatatctacgcatttcaccgctacactaggaattccactttcctctccgatactccagcctctcagtttccatcccatcacggggttaagccccgcacttttaagatggacttaagaagccgcctgcgcgcgctttacgcccaataattccggacaacgcttgccacctacgta

SEQ ID NO: 18 - DNA, 252 bp, Dialister invisus
cctgtttgctccccacgctttcgcgcctcagcgtcagttttcgtccagaaagtcgccttcgccaccggtgttcttcctaatctctacgcatttcaccgctacactaggaattccactttcctctccgatactccagcttcccagtttccttcccatcacggggttaagccccgcacttttaagagggacttgggaagccgcctgcgcgcgctttacgcccaataattccggacaacgcttgccacctacgta

SEQ ID NO: 19 - DNA, 252 bp, Dialister invisus
cctgtttgctccccacgctttcgagcctcaacgtcagttaccgtccagtaagccgccttcgccactggtgttcctcctaatatctacgcatttcaccgctacactaggaattccgcttacctctccgatactccagcttcccagtttccttcccatcacggggttaagccccgcacttttaagagggacttgggaagccgcctgcgcgcgctttacgcccaataattccggacaacgcttgccacctacgta

SEQ ID NO: 20 - DNA, 252 bp, Dialister propionifaciens
cctgtttgctacccacactttcgtgcctcagcgtcagttgtcgtccagaaagtcgccttcgccaccggtgttcttcctaatctctacgcatttcaccgctacactaggaattccactttcctctccgatactccagcctcccagtttccatcccatcacggggttaagccccgcacttttaagatggacttaagaagccgcctgcgcgcgctttacgcccaataattccggacaacgcttgccacctacgta

SEQ ID NO: 21 - DNA, 252 bp, Dialister succinatiphilus
cctgtttgctccccacgctttcgagcctcaacgtcagtcatcgtccagcaagccgccttcgccactggtgttcctcctaatatctacgcatttcaccgctacactaggaattccactttcctctccgatactccagctttccagtttccatcccatcacggggttaagccccgcacttttaagatggacttagaaagccgcctgcgcgcgctttacgcccaataattccggacaacgcttgccacctacgta

SEQ ID NO: 22 - DNA, 252 bp, Dialister invisus
cctgtttgctccccacgctttcgagcctcagcgtcagttaaagcccagtaagccgccttcgccactgatgttcctcctaatatctacgcatttcaccgctacactaggaattccactttcctctccgatactccagcttcccagtttccttcccatcacggggttaagccccgcacttttaagagggacttgggaagccgcctgcgcgcgctttacgcccaataattccggacaacgcttgccacctacgta

SEQ ID NO: 23 - DNA, 252 bp, Dialister pneumosintes
cccgttcgctcccctggctttcgcgcctcagcgtcagttttcgtccagaaagtcgccttcgccactggtgttcttcctaatatctacgcatttcaccgctacactaggaattccactttcctctccgatactccagcttcccagtttccatcccctcatggggttgagccccacgcttttaagatggacttaagaaaccgcctgcgcgcgctttacgcccaataattccggacaacgcttgccacctacgta

SEQ ID NO: 24 - DNA, 252 bp, Dialister pneumosintes
cctgtttgctccccacgctttcgcgcctcagcgtcagttttcgtctagaaagtcgccttcgccaccggtgttcttcctaatctctacgcatttcaccgctacactaggaattccactttcccctccgatactccagcttcccagtttccatcccctcatggggttgagccccacgcttttaagatggacttaagaaaccgcctgcgcgcgctttacgcccaataattccggacaacgcttgccacctacgta

SEQ ID NO: 25 - DNA, 19 bp, Artificial Sequence
  Primer
gtgccagcmgccgcggtaa

SEQ ID NO: 26 - DNA, 20 bp, Artificial Sequence
  Primer
ggactachvgggtwtctaat